European Patent Application EP 4 458 860 A1, published November 6, 2024. Title: Antibody specifically binding to acid sphingomyelinase and uses thereof. Applicant: Kyungpook National University Industry-Academic Cooperation Foundation. Application KR. The sequence listing filed with the application follows.

SEQUENCE LISTING (20 sequences)

SEQ ID NO: 1 - protein, 5 aa, synthetic construct
  REGION 1..5: note = 23A12C3 VH CDR1
DYYMN

SEQ ID NO: 2 - protein, 17 aa, synthetic construct
  REGION 1..17: note = 23A12C3 VH CDR2
VINPYNDGTSYNQKFKG

SEQ ID NO: 3 - protein, 14 aa, synthetic construct
  REGION 1..14: note = 23A12C3 VH CDR3
EKLYYYGRDYAMDY

SEQ ID NO: 4 - protein, 11 aa, synthetic construct
  REGION 1..11: note = 23A12C3 VL CDR1
RSSQDISNYLN

SEQ ID NO: 5 - protein, 7 aa, synthetic construct
  REGION 1..7: note = 23A12C3 VL CDR2
YTSRLHS

SEQ ID NO: 6 - protein, 9 aa, synthetic construct
  REGION 1..9: note = 23A12C3 VL CDR3
QQDNTLPYT

SEQ ID NO: 7 - DNA, 15 bp, synthetic construct
  misc_feature 1..15: note = 23A12C3 VH CDR1
  source 1..15: mol_type = other DNA
gactactatatgaac

SEQ ID NO: 8 - DNA, 51 bp, synthetic construct
  misc_feature 1..51: note = 23A12C3 VH CDR2
  source 1..51: mol_type = other DNA
gttattaatccttacaacgatggtactagctacaaccagaagttcaagggc

SEQ ID NO: 9 - DNA, 42 bp, synthetic construct
  misc_feature 1..42: note = 23A12C3 VH CDR3
  source 1..42: mol_type = other DNA
gagaagctttattactacggtagggactatgctatggactac

SEQ ID NO: 10 - DNA, 33 bp, synthetic construct
  misc_feature 1..33: note = 23A12C3 VL CDR1
  source 1..33: mol_type = other DNA
aggtcaagtcaggacattagcaattatttaaac

SEQ ID NO: 11 - DNA, 21 bp, synthetic construct
  misc_feature 1..21: note = 23A12C3 VL CDR2
  source 1..21: mol_type = other DNA
tacacatcaagattacactca

SEQ ID NO: 12 - DNA, 27 bp, synthetic construct
  misc_feature 1..27: note = 23A12C3 VL CDR3
  source 1..27: mol_type = other DNA
caacaggataatacgcttccgtacacg

SEQ ID NO: 13 - protein, 123 aa, synthetic construct
  REGION 1..123: note = 23A12C3 HC variable region
EVQLQQSGPVLVKPGASVKMSCKASGYTFTDYYMNWVKQSHGKSLEWIGVINPYNDGTSYNQKFKGKATLTVDKSSSTAYMELNSLTSEDSAVYYCAREKLYYYGRDYAMDYWGQGTSVTVSS

SEQ ID NO: 14 - protein, 466 aa, synthetic construct
  REGION 1..466: note = 23A12C3 HC
MGWSWIFLFLLSGTAGVHSEVQLQQSGPVLVKPGASVKMSCKASGYTFTDYYMNWVKQSHGKSLEWIGVINPYNDGTSYNQKFKGKATLTVDKSSSTAYMELNSLTSEDSAVYYCAREKLYYYGRDYAMDYWGQGTSVTVSSAKTTPPSVYPLAPGSAAQTNSMVTLGCLVKGYFPEPVTVTWNSGSLSSGVHTFPAVLQSDLYTLSSSVTVPSSTWPSQTVTCNVAHPASSTKVDKKIVPRDCGCKPCICTVPEVSSVFIFPPKPKDVLTITLTPKVTCVVVDISKDDPEVQFSWFVDDVEVHTAQTKPREEQINSTFRSVSELPIMHQDWLNGKEFKCRVNSAAFPAPIEKTISKTKGRPKAPQVYTIPPPKEQMAKDKVSLTCMITNFFPEDITVEWQWNGQPAENYKNTQPIMDTDGSYFVYSKLNVQKSNWEAGNTFTCSVLHEGLHNHHTEKSLSHSPGK

SEQ ID NO: 15 - protein, 107 aa, synthetic construct
  REGION 1..107: note = 23A12C3 LC variable region
DIQMTQTTSSLSASLGDRVTISCRSSQDISNYLNWCQQKPDGTVKLLIYYTSRLHSGVPSRFSGSGSGTDYSLTISNLEQEDIATYFCQQDNTLPYTFGGGTKLEIK

SEQ ID NO: 16 - protein, 233 aa, synthetic construct
  REGION 1..233: note = 23A12C3 LC
MSSAQFLGLLLLCFQGTRCDIQMTQTTSSLSASLGDRVTISCRSSQDISNYLNWCQQKPDGTVKLLIYYTSRLHSGVPSRFSGSGSGTDYSLTISNLEQEDIATYFCQQDNTLPYTFGGGTKLEIKRADAAPTVSIFPPSSEQLTSGGASVVCFLNNFYPKDINVKWKIDGSERQNGVLNSWTDQDSKDSTYSMSSTLTLTKDEYERHNSYTCEATHKTSTSPIVKSFNRNEC

SEQ ID NO: 17 - DNA, 369 bp, synthetic construct
  misc_feature 1..369: note = 23A12C3 HC variable region
  source 1..369: mol_type = other DNA
gaggtccagctgcaacagtctggacctgtgctggtgaagcctggggcttcagtgaagatgtcctgtaaggcttctggatacacattcactgactactatatgaactgggtgaaacagagccatggaaagagccttgagtggattggagttattaatccttacaacgatggtactagctacaaccagaagttcaagggcaaggccacattgactgttgacaagtcctccagcacagcctacatggagctcaacagcctgacatctgaggactctgcagtctattactgtgcaagagagaagctttattactacggtagggactatgctatggactactggggtcaaggaacctcagtcaccgtctcctca

SEQ ID NO: 18 - DNA, 1401 bp, synthetic construct
  misc_feature 1..1401: note = 23A12C3 HC
  source 1..1401: mol_type = other DNA
atgggatggagctggatctttctcttcctcctgtcaggaactgcaggtgtccactctgaggtccagctgcaacagtctggacctgtgctggtgaagcctggggcttcagtgaagatgtcctgtaaggcttctggatacacattcactgactactatatgaactgggtgaaacagagccatggaaagagccttgagtggattggagttattaatccttacaacgatggtactagctacaaccagaagttcaagggcaaggccacattgactgttgacaagtcctccagcacagcctacatggagctcaacagcctgacatctgaggactctgcagtctattactgtgcaagagagaagctttattactacggtagggactatgctatggactactggggtcaaggaacctcagtcaccgtctcctcagccaaaacgacacccccatctgtctatccactggcccctggatctgctgcccaaactaactccatggtgaccctgggatgcctggtcaagggctatttccctgagccagtgacagtgacctggaactctggatccctgtccagcggtgtgcacaccttcccagctgtcctgcagtctgacctctacactctgagcagctcagtgactgtcccctccagcacctggcccagccagaccgtcacctgcaacgttgcccacccggccagcagcaccaaggtggacaagaaaattgtgcccagggattgtggttgtaagccttgcatatgtacagtcccagaagtatcatctgtcttcatcttccccccaaagcccaaggatgtgctcaccattactctgactcctaaggtcacgtgtgttgtggtagacatcagcaaggatgatcccgaggtccagttcagctggtttgtagatgatgtggaggtgcacacagctcagacgaaaccccgggaggagcagatcaacagcactttccgttcagtcagtgaacttcccatcatgcaccaggactggctcaatggcaaggagttcaaatgcagggtcaacagtgcagctttccctgcccccatcgagaaaaccatctccaaaaccaaaggcagaccgaaggctccacaggtgtacaccattccacctcccaaggagcagatggccaaggataaagtcagtctgacctgcatgataacaaacttcttccctgaagacattactgtggagtggcagtggaatgggcagccagcggagaactacaagaacactcagcccatcatggacacagatggctcttacttcgtctacagcaagctcaatgtgcagaagagcaactgggaggcaggaaatactttcacctgctctgtgttacatgagggcctgcacaaccaccatactgagaagagcctctcccactctcctggtaaatga

SEQ ID NO: 19 - DNA, 321 bp, synthetic construct
  misc_feature 1..321: note = 23A12C3 LC variable region
  source 1..321: mol_type = other DNA
gatatccagatgacacagactacatcctccctgtctgcctctctgggagacagagtcaccatcagttgcaggtcaagtcaggacattagcaattatttaaactggtgtcagcagaaaccagatggaactgttaaactcctgatctactacacatcaagattacactcaggagtcccatcaagattcagtggcagtgggtctggaacagattattctctcaccattagcaacctggagcaagaagatattgccacttacttttgccaacaggataatacgcttccgtacacgttcggaggggggaccaagctggaaataaaa

SEQ ID NO: 20 - DNA, 702 bp, synthetic construct
  misc_feature 1..702: note = 23A12C3 LC
  source 1..702: mol_type = other DNA
atgtcctctgctcagttccttggtctcctgttgctctgttttcaaggtaccagatgtgatatccagatgacacagactacatcctccctgtctgcctctctgggagacagagtcaccatcagttgcaggtcaagtcaggacattagcaattatttaaactggtgtcagcagaaaccagatggaactgttaaactcctgatctactacacatcaagattacactcaggagtcccatcaagattcagtggcagtgggtctggaacagattattctctcaccattagcaacctggagcaagaagatattgccacttacttttgccaacaggataatacgcttccgtacacgttcggaggggggaccaagctggaaataaaacgggctgatgctgcaccaactgtatccatcttcccaccatccagtgagcagttaacatctggaggtgcctcagtcgtgtgcttcttgaacaacttctaccccaaagacatcaatgtcaagtggaagattgatggcagtgaacgacaaaatggcgtcctgaacagttggactgatcaggacagcaaagacagcacctacagcatgagcagcaccctcacgttgaccaaggacgagtatgaacgacataacagctatacctgtgaggccactcacaagacatcaacttcacccattgtcaagagcttcaacaggaatgagtgttag